European Patent Specification EP 3 376 852 B1, published June 4, 2025. Title: Rice grain with thickened aleurone. Applicant: Commonwealth Scientific and Industrial Research Organisation. The sequence listing filed with the application follows.

SEQUENCE LISTING (50 sequences)

SEQ ID NO: 1 - protein, 1959 aa, Artificial Sequence
  Rice ROS1a mutant (Ta2) polypeptide
MQDFGQWLPQSQTTADLYFSSIPIPSQFDTSIETQTRTSAVVSSEKESANSFVPHNGTGLVERISNDAGLTEVVGSSAGPTECIDLNKTPARKPKKKKHRPKVLKDDKPSKTPKSATPIPSTEKVEKPSGKRKYVRKKTSPGQPPAEQAASSHCRSELKSVKRSLDFGGEVLQESTQSGSQVPVAEICTGPKRQSIPSTIQRDSQSQLACHVVSSTSSIHTSASQMVNAHLFPPDNMPNGVLLDLNNSTSQLQNEHAKFVDSPARLFGSRIRQTSGKNSLLEIYAGMSDRNVPDLNSSISQTHSMSTDFAQYLLSSSQASVRETQMANQMLNGHRMPENPITPSHCIERAALKEHLNHVPHAKAAVMNGQMPHSYRLAQNPILPPNHIEGYQVMENLSELVTTNDYLTASPFSQTGAANRQHNIGDSMHIHALDPRRESNASSGSWISLGVNFNQQNNGWASAGAADAASSHAPYFSEPHKRMRTAYLNNYPNGVVGHFSTSSTDLSNNENENVASAINSNVFTLADAQRLIAREKSRASQRMISFRSSKNDMVNRSEMVHQHGRPAPHGSACRESIEVPDKQFGLMTEELTQLPSMPNNPQREKYIPQTGSCQLQSLEHDMVKGHNLAGELHKQVTSPQVVIQSNFCVTPPDVLGRRTSGEHLRTLIAPTHASTCKDTLKALSCQLESSRDIIRPPVNPIGPSSADVPRTDNHQVKVSEETVTAKLPEKRKVGRPRKELKPGEKPKPRGRPRKGKVVGGELASKDSHTNPLQNESTSCSYGPYAGEASVGRAVKANRVGENISGAMVSLLDSLDIVIQKIKVLDINKSEDPVTAEPHGALVPYNGEFGPIVPFEGKVKRKRSRAKVDLDPVTALMWKLLMGPDMSDCAEGMDKDKEKWLNEERKIFQGRVDSFIARMHLVQGDRRFSPWKGSVVDSVVGVFLTQNVSDHLSSSAFMALAAKFPVKPEASEKPANVMFHTISENGDCSGLFGNSVKLQGEILVQEASNTAASFITTEDKEGSNSVELLGSSFGDGVDGAAGVYSNIYENLPARLHATRRPVVQTGNAVEAEDGSLEGVVSSENSTISSQNSSDYLFHMSDHMFSSMLLNFTAEDIGSRNMPKATRTTYTELLRMQELKNKSNETIESSEYHGVPVSCSNNIQVLNGIQNIGSKHQPLHSSISYHQTGQVHLPDIVHASDLEQSVYTGLNRVLDSNVTQTSYYPSPHPGIACNNETQKADSLSNMLYGIDRSDKTTSLSEPTPRIDNCFQPLSSEKMSFAREQSSSENYLSRNEAEAAFVKQHGTSNVQGDNTVRTEQNGGENSQSGYSQQDDNVGFQTATTSNLYSSNLCQNQKANSEVLHGVSSNLIENSKDDKKTSPKVPVDGSKAKRPRVGAGKKKTYDWDMLRKEVLYSHGNKERSQNAKDSIDWETIRQAEVKEISDTIRERGMNNMLAERIKDFLNRLVRDHGSIDLEWLRYVDSDKAKDYLLSIRGLGLKSVECVRLLTLHHMAFPVDTNVGRICVRLGWVPLQPLPESLQLHLLEMYPMLENIQKYLWPRLCKLDQRTLYELHYQMITFGKVFCTKSKPNCNACPMRAECKHFASAFASARLALPGPEEKSLVTSGTPIAAETFHQTYISSRPVVSQLEWNSNTCHHGMNNRQPIIEEPASPEPEHETEEMKECAIEDSFVDDPEEIPTIKLNFEEFTQNLKSYMQANNIEIEDADMSKALVAITPEVASIPTPKLKNVSRLRTEHQVYELPDSHPLLEGFNQREPDDPCPYLLSIWTPGETAQSTDAPKSVCNSQENGELCASNTCFSCNSIREAQAQKVRGTLLIPCRTAMRGSFPLNGTYFQVNECSNVMRQVFADHDSSRNPIDVPRSWIWNLPRRTVYFGTSIPTIFKGLTTEEIQHCFWRGFVCVRGFDRTSRAPRPLYARLHFPASKITRNKKSAGSAPGRDDE

SEQ ID NO: 2 - protein, 1952 aa, Oryza sativa
MQDFGQWLPQSQTTADLYFSSIPIPSQFDTSIETQTRTSAVVSSEKESANSFVPHNGTGLVERISNDAGLTEVVGSSAGPTECIDLNKTPARKPKKKKHRPKVLKDDKPSKTPKSATPIPSTEKVEKPSGKRKYVRKKTSPGQPPAEQAASSHCRSELKSVKRSLDFGGEVLQESTQSGSQVPVAEICTGPKRQSIPSTIQRDSQSQLACHVVSSTSSIHTSASQMVNAHLFPPDNMPNGVLLDLNNSTSQLQNEHAKFVDSPARLFGSRIRQTSGKNSLLEIYAGMSDRNVPDLNSSISQTHSMSTDFAQYLLSSSQASVRETQMANQMLNGHRMPENPITPSHCIERAALKEHLNHVPHAKAAVMNGQMPHSYRLAQNPILPPNHIEGYQVMENLSELVTTNDYLTASPFSQTGAANRQHNIGDSMHIHALDPRRESNASSGSWISLGVNFNQQNNGWASAGAADAASSHAPYFSEPHKRMRTAYLNNYPNGVVGHFSTSSTDLSNNENENVASAINSNVFTLADAQRLIAREKSRASQRMISFRSSKNDMVNRSEMVHQHGRPAPHGSACRESIEVPDKQFGLMTEELTQLPSMPNNPQREKYIPQTGSCQLQSLEHDMVKGHNLAGELHKQVTSPQVVIQSNFCVTPPDVLGRRTSGEHLRTLIAPTHASTCKDTLKALSCQLESSRDIIRPPVNPIGPSSADVPRTDNHQVKVSEETVTAKLPEKRKVGRPRKELKPGEKPKPRGRPRKGKVVGGELASKDSHTNPLQNESTSCSYGPYAGEASVGRAVKANRVGENISGAMVSLLDSLDIVIQKIKVLDINKSEDPVTAEPHGALVPYNGEFGPIVPFEGKVKRKRSRAKVDLDPVTALMWKLLMGPDMSDCAEGMDKDKEKWLNEERKIFQGRVDSFIARMHLVQGDRRFSPWKGSVVDSVVGVFLTQNVSDHLSSSAFMALAAKFPVKPEASEKPANVMFHTISENGDCSGLFGNSVKLQGEILVQEASNTAASFITTEDKEGSNSVELLGSSFGDGVDGAAGVYSNIYENLPARLHATRRPVVQTGNAVEAEDGSLEGVVSSENSTISSQNSSDYLFHMSDHMFSSMLLNFTAEDIGSRNMPKATRTTYTELLRMQELKNKSNETIESSEYHGVPVSCSNNIQVLNGIQNIGSKHQPLHSSISYHQTGQVHLPDIVHASDLEQSVYTGLNRVLDSNVTQTSYYPSPHPGIACNNETQKADSLSNMLYGIDRSDKTTSLSEPTPRIDNCFQPLSSEKMSFAREQSSSENYLSRNEAEAAFVKQHGTSNVQGDNTVRTEQNGGENSQSGYSQQDDNVGFQTATTSNLYSSNLCQNQKANSEVLHGVSSNLIENSKDDKKTSPKVPVDGSKAKRPRVGAGKKKTYDWDMLRKEVLYSHGNKERSQNAKDSIDWETIRQAEVKEISDTIRERGMNNMLAERIKDFLNRLVRDHGSIDLEWLRYVDSDKAKDYLLSIRGLGLKSVECVRLLTLHHMAFPVDTNVGRICVRLGWVPLQPLPESLQLHLLEMYPMLENIQKYLWPRLCKLDQRTLYELHYQMITFGKVFCTKSKPNCNACPMRAECKHFASAFASARLALPGPEEKSLVTSGTPIAAETFHQTYISSRPVVSQLEWNSNTCHHGMNNRQPIIEEPASPEPEHETEEMKECAIEDSFVDDPEEIPTIKLNFEEFTQNLKSYMQANNIEIEDADMSKALVAITPEVASIPTPKLKNVSRLRTEHQVYELPDSHPLLEGFNQREPDDPCPYLLSIWTPGETAQSTDAPKSVCNSQENGELCASNTCFSCNSIREAQAQKVRGTLLIPCRTAMRGSFPLNGTYFQVNEVFADHDSSRNPIDVPRSWIWNLPRRTVYFGTSIPTIFKGLTTEEIQHCFWRGFVCVRGFDRTSRAPRPLYARLHFPASKITRNKKSAGSAPGRDDE

SEQ ID NO: 3 - protein, 1636 aa, Oryza sativa
MEGQWLHEPHGINLCFSTSSTLPRMNPSIETGTRNVTHVPSKNVSTSSSQARKTTVQKPKRKRHRPKVIKEGKATQAHKSTTSEPPKEKDKPAGKRKYVRRKEQNTTPTEHHPPSKDAVAHTIVVPTLAKRCFNFDGRDHHEENVDLLSQTRVEETPTCYGDAQLLTSAVDGSNIQLVQPWCGIGSPIFASVDPMANMRQIWAESSRANRVTFDLNNSAVNHIPRRFSNPTNSYGQNFQFGSREQINQYQHFYDDDIPDEIPENLVVPAWHTGRTWMVGNFNHEASTRVVNPMPQGYRVPQSPSEPPTCSERNTTNINLSEFPAKNDQSKFATNPNDQIGASFGLCDSHFSDVHAIGKKRGYDTITDHQVSFDAYLEQSNSRRQFYSDPLSTSSETYLLTETCKRMRSENHSSWLDGFIGNVSSTSANLSGNWNTNNVLAINHGVCTTLADVQRSMALEESRSSRQYTDPTLPCTSNTHFIGSCAQHTNSPDSAMNSLGENIGHRNGDHQLESLEIRPTQHYTSECLGLPNEWSGHLSAGHTHLPNETMIPSINKNWSCSVAWAASAAQPTATVSQVASAAAATSTAQPSEQRDYIPSSGVHQPQPLENQMVKGQDLCQTHKTSTKYVADGNPSINTPVEHIQRTPIEVMSSFQSVNRPATTKNCHLEASRETTSANPTEKPKVWSRPRKEVEPVGKPKARGHPKKQAEPDEKPKARGRVRKTTEANGKAEDRDPTMKENDEAIIEKLKLLSINMTSNNTVEETPKDLGALVPLEGKVKKRGSRAEVKIDPVTNLMWNLLMALDKCEGVEGIDEDKERLLEEERRMFRGRIDSFIAHMHLVQGDRRFSPWKGSIVDSVVDVFLTQNVSDHLSSSAFMALAARFPVKSEGPEKPAAVEKSTPTPPKQKDSCSGVLGESAKLQGNFFVEEIGDLGSFNTVDDGSLEGVLSSQNSVVSPRNFSKYLLNGTYTMGSSSSLVKFTQEVGSSGCHQVSVLPTSDLNKAAPFDLDTTYQICTGLDHGVNISDVAQSEVSLYQQHPIDASINKNKAKVTDYSSGSFLYDNRDGSLSQHMYSSFPFQPSQEAECSATVKQSFFQQFISSEEVPISTGHSFYDNSFTSNRTEDPYVEQQDCFNNLQEAYTTRTIQINSERSQPECSQQQDNDIRVQAKTCEKHSSSNLCGNMNSHSDVPLGIASGSIGKSKHTEKRPKARNVRGRTKMKHYDWDNLRKEVLHNHGNRQRSDKAKDTIDWEADFLNRLVRDHGSIDLEWLRDIEPDKAKGFLLSIRGLGLKSTECVRLLTLHQMAFPVDTNVARICVRLGWVPLQPLPESLQLHLLELYPLLEHIQKYIWPRLCKLDQLILYELHYQMITFGKVFCSKSKPNCNSCPMRAECKHFASAFASARLALPGPSKKTSKPEYPNDAESSHKKYTHSRPMGQLSWNTNHPGHVYEAREAEIEDFFSEDPDEIPIINLNVEEFAQNLKSYIHANNIEIEDADMSNALVAISPQAASVPTSKLKNVNRLRTEHQVYELPDSHPLLEGFDQREPDDPSPYLLSIWTPGKLMCSHPTFTLIQVILMIKISTGETAQSTDAPKTFCNSKETGKLCESSTCFSCNSTREMQSQKVRGTLLASSLLRVP

SEQ ID NO: 4 - protein, 1847 aa, Oryza sativa
MAKDENPSYLHLIFLSSRIRVFILDPPLSLPLSHGQCELQVVEEAAMDPSGLNLQGNPAENQESWTSGVSVGRGTPNLGVGTAVAGRSCPSSTLFPGSSLSSTALLNTMHEGSFPQTALVAGSVSSADEQHGAPPVRPSYNLPAGCTQVPISILVFHRRLTGRGSRCRSPQSRSFMPAPALSGVSEDGAYGPIPQSDFLSLRGPSEVFPGDMAMNHSEPATSYGYNSEYAPMHLQPNGLYTEASNTESEREASQLQQSAEAVICDSLSKLESAMEKIQGQNPQESSGLVAEGSADDNIHKYHQKAKRARTQITHSDKIDLPTQAVSACKEKTITQIEMQIADAERTEALKGEDAPAQKLKTRRRKHRPKVIREDRPAKKQMATTSEEKPLNQKPKRKYVRKNRNPSSLEKCAEPFSDHSISRESRTTVRSSIASVRRRLQFEFGEHGVQRDQSSMTNSWYQNQEKPVNAESSLCSVTKSSVQVEHGQELHMENSPEGLFFGINSKLNKILDEYIHLPEAAPKPSEQIPLAASGHVSEELARKQYDVRHTHDPDSTSYNIERSGLITTKGHKKDLDLNYSNTNGFQMYCSASLLPEMDSTKGSMTKVSKMDKNKKRHYGGESSLAGTQSSIIMRTAAEMLAVYQACGIKKKRSARVRRNSFLSVMDLEKNTSQESTRLPRSCMEALYESSYIKFMTKKRSQKARLNSPNSIQPNIDQKNRFSSETVFSGGFNGLKRSEETFQKTLPQIPDDKRINLDIHCKVPVESSPNTSTPPYMDYLQGVTSKFRYFDLNTEQVHKTEMHLSQTMPSLSSLGATNYLPNALVPYVGGAVVPYQTQFHLVKKQRPRAKVDLDFETTRVWNLLMGKAADPVDGTDVDKERWWKQEREVFQGRANSFIARMRLVQGDRRFSPWKGSVVDSVVGVFLTQNVADHLSSSAYMALAASFPTGSHGNCNDGIAGQDNEEIISTSAVGDRGTFEFFYNGSRPDIGLNFEFSMACEKIHMEPKDNTTVNELTKGENYSLHCKESAGSLCDHETEIDHKAKSISDFSAVELTACMKNLHATQFQKEISLSQSVVTSESILQPGLPLSSGMDHARRNFVGSISDTASQQVGSNFDDGKSLTGNDVTANETEYHGIKAAATNNYVVDEPGIPSGSSLYPFFSAIDCHQLDGRNDTHVSSTSPNCSICSASSNFKIGTIEENSSLFMPFDAHLAQRNGNMIVDTNLSSALESTELPVKLLHCGKRSCYEASEFQDHESLYATGGVIPETATKADDSTLKSGFASFNGLPDTAAQASKPKKSRTTSKKNSENFDWDKLRRQACGNYQMKERIFDRRDSVDWEAVRCADVQRISHAIRERGMNNVLAERIQKFLNRLVTDHGSIDLEWLRDVPPDSAKDYLLSIRGLGLKSVECVRLLTLHHLAFPVDTNVGRICVRLGWVPIQPLPESLQLHLLELYPVLETIQKYLWPRLCKLDQQTLYELHYQMITFGKVFCTKSKPNCNACPMRSECRHFASAFASARLALPSPQDKRLVNLSNQFAFHNGTMPTPNSTPLPQLEGSIHARDVHANNTNPIIEEPASPREEECRELLENDIEDFDEDTDEIPIIKLNMEAFSQNLENCIKESNKDFQSDDITKALVAISNEAASIPVPKLKNVHRLRTEHYVYELPDSHPLMQQLALDQREPDDPNELKDTREAPKPCCNPQTEGGLCSNEMCHNCVSERENQYRYVRGTVLVPCRTAMRGSFPLNGTYFQVNEVFADHSSSHNPINIPREQLWNLHRRMVYFGTSVPTIFKGLTTEEIQHCFWRGFVCVRGFNMETRAPRPLCPHFHLAASKLRRSSKKAATEQTH

SEQ ID NO: 5 - protein, 1829 aa, Oryza sativa
MAKDENPSYLHLIFLSSRIRVFILDPPHSLSLSNGQCELQVVEEAAMDPSGLNLQGNPAENQESWTSGVSVGRGTPNLGVGTAVAGRSCPPLTLFPGSSLSSTALLNAMHEGSFPQAALVAGSGSSADEQHGGPPVRPSYNLPAGCTQVPISILVFHRRLTGRGSRRRSFMPAPALSGVSEDGASGPIPQSDFLSLGGPSEVFAEHAPMLLQPNGLYTEASNTESEREASQLQQSAEAVICDSHSKLESVMEKIQGQNPQESIGLVAEGSTDDNIHKYHQKAKRARTQITHSDKMDLPTQAVSACKEKTLTQIEMQIADAERTEAFKSEDAPAQKLKTRRRKHRPKVIREDRPAKKQMSTTSKEKPLNQKPKRKYVWKNRNPSSLEKCAEPFSDHSISRESRTTVRSSIASVRRRLQFEFGEHGVQRDQSSRTNSWYRNQEKPVNAESSLCSVTKSSVQVEHGQELHMENSPEGLFFGINSKLNKILDEYIHLPEAAPKPSEEIPLATSGHVSEELARKQDDVRHIHDHNERSGLITTKQNKKDLDLNYSNTNGFQMYCSASLLPEMDSTKGRMTKVSKMDKNQKRHYGGESSLAGTQSSIIMRTAAEMLAVYQACGIKKKRSARVRRNSFLSVMDLEKNTSQESTRLPRSCMEALYESSYIKFMTKKRSQKARLNSPNSIQPNIDQKNRFSSETIFSGGFNGLKRSEETFQKTLPQIPDDKRINLDIHCEVPVENSPNTSTPPYMDYLQGVTSKFRYFDLNTEQVHKTEMHLYQTMPSLSSLGATNYLPNALVPYVGGAVVPYQTQFHLVKKQRPRAKVDLDFETTRVWNLLMGKAADPVDGTDVDKERWWKQEREVFQGRANSFIARMRLVQGDRRFSPWKGSVVDSVVGVFLTQNVADHLSSSAYMALAASFPPGSDGNCNDGIAGQDNEEIISTSAVRDRGTFEFFYDGSRPDIGLNFEELSMACEKIHMEPKGNATVNELTKGENYSLHCKEPAGSLCDHETRIDHKAKSISDISLVELTARMKNLHATQFQTEISLSQSVVTSESILQPGLPLSSGMDHAPRNFVGGISDTASQQVGSNFDDGKSLTGNDVTANETEYHGIKAAATNNYVVDEPRIPSGSNMYPFFSATDCHQLDERNDIHVSSTSPNSSIGSASSNFKIGTIEENSSFFMPFDAHLAQMNGNMIAGTNVSSALASTELPVKLLHCCKRSCYEASEFQDHESLYATGGAIPETATKADDSTLKSGFASFNGLPDTAAQASKPKKPRTTSKKNSENFDWDKLRRQACGNYQMKERIFDRRDSVDWEAVRCADVQRISHAIRERGMNNVLAERIQKFLNRLVTDHGSIDLEWLRDVPPDSAKDYLLSIRGLGLKSVECVRLLTLHHLAFPVDTNVGRICVRLGWVPIQPLPESLQLHLLELYPVLETIQKYLWPRLCKLDQQTLYELHYQMITFGKVFCTKSKPNCNACPMRSECKHFASAFASARLALPSPQDKRLVNMSNQFDFQNGTMPTPHSTPLLQLEGSIHARDVHANNTNPIIEEPASPREEECRELLENDIEDFDEDTDEIPTIKLNMEAFAQNLENCIKESNKDFQSDDITKALVAISNEAASIPVPKLKNVHRLRTEHYVYELPDSHPLMQQLALDQREPDDPSPYLLAIWTPDELKDTREAPKPCCNPQTEGGLCSNEMCHNCVSERENQYRYVRGTVLVPCRTAMRGSFPLNGTYFQVNEVFADHSSSHNPINIPREQLWNLHRRMVYFGTSVPTIFKGLTTEEIQHCFWRGFVCVRGFDMETRAPRPLCPHFHLAASKLRRSSKTAATEQTH

SEQ ID NO: 6 - protein, 1987 aa, Arabidopsis thaliana
MNSRADPGDRYFRVPLENQTQQEFMGSWIPFTPKKPRSSLMVDERVINQDLNGFPGGEFVDRGFCNTGVDHNGVFDHGAHQGVTNLSMMINSLAGSHAQAWSNSERDLLGRSEVTSPLAPVIRNTTGNVEPVNGNFTSDVGMVNGPFTQSGTSQAGYNEFELDDLLNPDQMPFSFTSLLSGGDSLFKVRQYGPPACNKPLYNLNSPIRREAVGSVCESSFQYVPSTPSLFRTGEKTGFLEQIVTTTGHEIPEPKSDKSMQSIMDSSAVNATEATEQNDGSRQDVLEFDLNKTPQQKPSKRKRKFMPKVVVEGKPKRKPRKPAELPKVVVEGKPKRKPRKAATQEKVKSKETGSAKKKNLKESATKKPANVGDMSNKSPEVTLKSCRKALNFDLENPGDARQGDSESEIVQNSSGANSFSEIRDAIGGTNGSFLDSVSQIDKTNGLGAMNQPLEVSMGNQPDKLSTGAKLARDQQPDLLTRNQQCQFPVATQNTQFPMENQQAWLQMKNQLIGFPFGNQQPRMTIRNQQPCLAMGNQQPMYLIGTPRPALVSGNQQLGGPQGNKRPIFLNHQTCLPAGNQLYGSPTDMHQLVMSTGGQQHGLLIKNQQPGSLIRGQQPCVPLIDQQPATPKGFTHLNQMVATSMSSPGLRPHSQSQVPTTYLHVESVSRILNGTTGTCQRSRAPAYDSLQQDIHQGNKYILSHEISNGNGCKKALPQNSSLPTPIMAKLEEARGSKRQYHRAMGQTEKHDLNLAQQIAQSQDVERHNSSTCVEYLDAAKKTKIQKVVQENLHGMPPEVIEIEDDPTDGARKGKNTASISKGASKGNSSPVKKTAEKEKCIVPKTPAKKGRAGRKKSVPPPAHASEIQLWQPTPPKTPLSRSKPKGKGRKSIQDSGKARGPSGELLCQDSIAEIIYRMQNLYLGDKEREQEQNAMVLYKGDGALVPYESKKRKPRPKVDIDDETTRIWNLLMGKGDEKEGDEEKDKKKEKWWEEERRVFRGRADSFIARMHLVQGDRRFSPWKGSVVDSVIGVFLTQNVSDHLSSSAFMSLAARFPPKLSSSREDERNVRSVVVEDPEGCILNLNEIPSWQEKVQHPSDMEVSGVDSGSKEQLRDCSNSGIERFNFLEKSIQNLEEEVLSSQDSFDPAIFQSCGRVGSCSCSKSDAEFPTTRCETKTVSGTSQSVQTGSPNLSDEICLQGNERPHLYEGSGDVQKQETTNVAQKKPDLEKTMNWKDSVCFGQPRNDTNWQTTPSSSYEQCATRQPHVLDIEDFGMQGEGLGYSWMSISPRVDRVKNKNVPRRFFRQGGSVPREFTGQIIPSTPHELPGMGLSGSSSAVQEHQDDTQHNQQDEMNKASHLQKTFLDLLNSSEECLTRQSSTKQNITDGCLPRDRTAEDVVDPLSNNSSLQNILVESNSSNKEQTAVEYKETNATILREMKGTLADGKKPTSQWDSLRKDVEGNEGRQERNKNNMDSIDYEAIRRASISEISEAIKERGMNNMLAVRIKDFLERIVKDHGGIDLEWLRESPPDKAKDYLLSIRGLGLKSVECVRLLTLHNLAFPVDTNVGRIAVRMGWVPLQPLPESLQLHLLELYPVLESIQKFLWPRLCKLDQRTLYELHYQLITFGKVFCTKSRPNCNACPMRGECRHFASAYASARLALPAPEERSLTSATIPVPPESYPPVAIPMIELPLPLEKSLASGAPSNRENCEPIIEEPASPGQECTEITESDIEDAYYNEDPDEIPTIKLNIEQFGMTLREHMERNMELQEGDMSKALVALHPTTTSIPTPKLKNISRLRTEHQVYELPDSHRLLDGMDKREPDDPSPYLLAIWTPGETANSAQPPEQKCGGKASGKMCFDETCSECNSLREANSQTVRGTLLIPCRTAMRGSFPLNGTYFQVNELFADHESSLKPIDVPRDWIWDLPRRTVYFGTSVTSIFRGLSTEQIQFCFWKGFVCVRGFEQKTRAPRPLMARLHFPASKLKNNKT

SEQ ID NO: 7 - DNA, 6835 bp, Artificial Sequence
  Full length cDNA encoding rice ROS1a mutant (Ta2) polypeptide
atgatagtgcatatgtatcctttctttttcttttcttttgttttcataactgtcttacagaatttcatgttggctggtgacacttgtctcactcattatttggtatattttgactaaatgcaacgtgttggtgctcggtagtttatatttgtttttacgcattcttcattgactgtatgtatttgatgttgataccctgggctgtcttattttataggtggatgctgggaggccacataggaggcctgtgtgatccaagtgtgctgctcctgagttgaaattgcatagccatatagcaactactggtgtaaacttgagagatgaagtagtgaaaggaaatatgcaggattttggacaatggctgcctcaatctcagaccactgccgatctatatttctccagtattccaataccatcacagttcgatacttccatagagacgcagactagaacttctgcagttgtatcgtcagagaaagaatctgctaattcgttcgtccctcataatggtactgggcttgttgaacgcattagcaatgatgctgggctaactgaagtagttggaagtagtgctggaccaactgaatgtattgacttgaacaagacaccagcacggaaacccaagaagaaaaagcacaggccaaaggtgctaaaggacgataaaccatcgaagacacctaaatctgctactccaataccttcaacagaaaaggtagaaaaaccatctggaaagagaaaatatgtccgcaagaagacatctccaggccaacctcctgcagaacaggcagctagctcacactgcagatctgagctgaagtcagttaaacgaagtttggactttggtggagaagtactgcaagagagtacacaatctggatctcaagttccggtggcagaaatatgtactggtcccaagcgtcaatcaataccttctaccatccaaagagattcgcaaagccagttggcttgccacgtggtttctagcaccagctcaattcacacttcagctagtcagatggttaatgcacatttgtttcctcctgataacatgccaaatggagtattgcttgacctcaataattctactagtcagttacaaaacgaacatgctaaatttgtggacagtccggcacgtctttttggttccagaataagacagacatcaggtaaaaattctttgctagaaatctatgctggcatgtcagatagaaatgtacctgatctcaacagttcaatcagtcagacgcatagcatgtctactgattttgctcaatacttgctttcatcctcacaagcttctgtaagggaaacacaaatggccaatcagatgcttaatggtcataggatgccagaaaatccaattacacctagtcattgtattgaaagggctgcattgaaggaacatttgaatcatgttcctcacgcaaaagccgcagtgatgaatggccaaatgccccatagttacaggttggcgcaaaatcccatcctacctccaaatcatattgaagggtatcaagtgatggaaaatttgagtgaacttgtcacgacaaatgactatctaactgctagtcctttcagtcaaactggagctgcaaataggcagcataatattggtgactccatgcatatacatgcattggatcctagaagagagagtaatgcttcaagtggttcttggatatcattaggtgtgaactttaaccaacaaaataatggatgggcatctgcaggtgctgccgatgctgcgagctcacatgccccatatttttcagaacctcacaaaagaatgaggacagcttatcttaacaattatccaaatggagtcgtgggacatttttctacctcatctacggatttgtcaaataatgagaatgaaaatgtggcctcagcaatcaactcaaacgtttttacccttgctgatgcacaaagattgatagcccgtgagaaatcacgagcttcccaaagaatgatcagttttagatcatctaaaaatgatatggttaacagatcagaaatggtccatcaacatggcagacctgctccgcatggctctgcatgcagggagtctattgaagtacctgacaaacagttcgggctcatgacagaagaactcacacaattacctagtatgccaaataacccacaaagggaaaaatatattccgcaaactggaagttgccaacttcagtctttggaacatgacatggttaaagggcataacttggcaggtgaattgcataagcaagtaacttcacctcaagttgttattcagagcaatttctgtgttacccctcctgatgtgctcggcagaagaaccagtggggagcatttaagaacccttatagctccaacacatgcatcgacatgtaaggacactctgaaagctttaagttgtcaactggagagttctagagacattattaggcctcctgtcaatcctatagggccatcctctgccgatgttccaagaactgataaccatcaagtcaaggtttctgaagaaaccgttacagccaaactccctgagaagcgaaaagtaggacgtcccagaaaagagttaaaacctggtgagaaaccaaaacctagaggccgtccaaggaagggaaaagttgttggtggagaacttgcatcaaaggatagtcacactaatccattgcaaaatgagagtacttcatgttcttatggtccttatgcaggggaggcttctgttggaagagcagttaaagcaaatagagttggagaaaacatttctggagctatggtatccctactggattctttagatattgttattcaaaagataaaggtcttggacataaacaaatcagaagaccctgtgacagctgaacctcatggtgctcttgtcccttacaatggagaatttggtcctattgttccttttgaggggaaagtgaaaagaaaacgctctcgagccaaagtggatcttgaccctgtaactgctttaatgtggaagttactaatgggaccagatatgagtgattgtgctgaaggtatggataaggataaagagaaatggctaaatgaagaaagaaaaatattccaagggcgtgttgattcatttattgctcgaatgcatctagttcaaggagatcggcgtttttctccttggaaaggatcagttgtagattctgtagtgggagtatttcttacacagaatgtttcggaccatctttccagctctgcatttatggctcttgctgcaaaatttcctgtaaagccagaagcctctgaaaaacccgcaaatgtgatgtttcatacaatttcagaaaatggtgattgttctgggttgtttggtaattctgtcaagctacagggtgagatccttgttcaggaggccagcaacacagcagcctcttttatcacaaccgaggataaggaaggaagtaacagtgtggaattgcttggaagttcttttggggatggagtggatggtgcagcaggagtttattctaatatttatgagaatctgccagctagactgcatgctactaggcgtccagtcgttcaaactggaaacgctgtcgaagcggaagatgggtcactggagggtgttgtttcatcagaaaactccactatttcatctcaaaattcatcagattatctatttcacatgtctgatcatatgttttcgagcatgttactaaatttcactgccgaagacattggcagcagaaatatgcccaaagcaacaagaaccacatatacagaacttctacgaatgcaggagctgaagaacaagtctaatgaaaccattgaatcatcagagtatcatggggttccagtctcatgtagtaacaacattcaagtgctcaatggaatacaaaatatcggcagtaaacatcagcctttacattcctctatttcatatcaccagactggccaagttcacctcccagacatagtacatgcgagtgatttggagcaatcagtatacactggccttaatagagtgcttgattctaatgttacacaaaccagttattatccttcacctcatcctggaattgcctgtaacaatgaaacacaaaaggctgactctttaagcaacatgttatatggtatagatagatcagataagactacttccctgtctgagcctacaccaagaatcgataactgttttcaaccattaagttcagagaaaatgtcatttgctagggaacagtcctcttctgaaaattatctttcaaggaatgaagctgaagctgcatttgttaaacagcatggaacatcaaatgtgcaaggtgataatactgtcaggacagagcaaaatggaggtgaaaattctcaatcaggatacagccaacaggatgataatgttggatttcaaacagcgacaaccagtaatctttattcttcaaacttatgccaaaaccagaaagcaaattctgaagtactacacggagtttcttccaacttgatagagaattctaaagatgacaaaaagacttcccccaaagttccagtcgatggatcaaaagcaaagaggccaagagttggggctggtaaaaagaaaacatatgattgggatatgttgagaaaagaagttctttacagtcatggtaataaagaaagatcccagaatgctaaggactcaattgattgggaaacaataagacaagcagaggtgaaggaaatatctgacacaattagagagcgaggaatgaataacatgctggcagaacggataaaagacttcctaaaccgattggtgagagaccatgggagcatcgatcttgagtggttgcgctatgtcgattcagataaagcgaaggactatctcttaagcattagaggacttggacttaaaagtgttgagtgtgtgcgtcttttgacactccatcacatggcttttcctgtggatacaaatgttggtagaatatgtgtgaggcttggatgggtgccacttcagcccctacccgagtctcttcagttgcacctgttggagatgtatccaatgctggagaacatacagaaatacctctggccgaggttatgcaagcttgatcaacggacattgtatgagcttcactatcaaatgataacttttggaaaggtattttgtacaaaaagtaagcccaattgcaacgcatgcccaatgagagctgagtgcaagcactttgcaagtgcatttgccagtgcaaggctcgctcttcctggacctgaagagaagagtttagttacatctggaaccccaatagctgcagaaaccttccaccagacatatataagttctaggcctgtagtaagtcagcttgagtggaattcaaacacctgtcaccatggtatgaacaatcgccagccaatcattgaggagccagcaagcccagaacctgaacatgagacagaagagatgaaagagtgtgcaatagaggatagttttgtcgatgatccagaagaaatccctactatcaagcttaattttgaggagtttacacagaacctgaagagttatatgcaagcaaataacattgagattgaagatgctgatatgtcaaaggctttggtcgctataactcctgaagttgcttctatcccaactcctaagctcaagaatgtcagtcgcctaaggacagagcaccaagtctatgaactgccagattcacatccacttcttgaaggattcaaccaaagagaaccagatgatccttgcccatacctactctctatatggaccccaggtgaaacagctcaatcaactgatgcacctaagtcggtctgcaattcacaagagaatggtgaactatgtgcaagcaatacatgctttagttgcaacagtataagagaagcgcaggcccaaaaagttcgagggacactgctgataccatgccgaacagcaatgagaggaagctttccacttaatgggacatattttcaagtcaatgagtgttcaaatgttatgcggcaggtatttgctgatcatgactcaagccggaacccgattgatgttccaaggagttggatatggaatctccctaggagaactgtttactttggaacttcaattccgacaatatttaaaggtttgacaactgaagaaatacaacattgcttttggagaggatttgtgtgcgtgagaggctttgataggacatcaagagcacccagaccactgtatgcaagactccactttccagcaagcaaaattaccaggaataaaaaatctgcaggttctgctccaggaagagatgatgaataggccatctggaaaaccagaaaggaaataaagaggaggtacatatgatctgccagaagatcactgacctgaaatggatcgctgaccaataagttgccgtaggcaattcaattatttctggccatatacatctgctgaaagttatgaactccagccactgacgaattcgtggtgctggtattcttcggcaacatgatccatcatacagattctatgcttggttgttgcaagcaattcttatgcggtgacagttgctgctgatagggagaaaaggcatgtccggcggctcagcggctctaactgtactttcatatgagtggaaccgattgttgtacatgtgaaaagtttgccattcaaaatggtcattcatgttgttaggtcattcatgtagtcgatgtcaaattaatcatcaattatttgatttgattcattcacaagtttaattggctctagatacttgtgagctgcaggccagcaatgtcataatgtatgtcgggaaaaggtagatataaatcgtcagcatttacctgaaatacccttcctctgtccataaatacaagggattttgggttgttaagcgtattttaagttcgatatgaaaattactttgatgttccg

SEQ ID NO: 8 - DNA, 6814 bp, Oryza sativa
atgatagtgcatatgtatcctttctttttcttttcttttgttttcataactgtcttacagaatttcatgttggctggtgacacttgtctcactcattatttggtatattttgactaaatgcaacgtgttggtgctcggtagtttatatttgtttttacgcattcttcattgactgtatgtatttgatgttgataccctgggctgtcttattttataggtggatgctgggaggccacataggaggcctgtgtgatccaagtgtgctgctcctgagttgaaattgcatagccatatagcaactactggtgtaaacttgagagatgaagtagtgaaaggaaatatgcaggattttggacaatggctgcctcaatctcagaccactgccgatctatatttctccagtattccaataccatcacagttcgatacttccatagagacgcagactagaacttctgcagttgtatcgtcagagaaagaatctgctaattcgttcgtccctcataatggtactgggcttgttgaacgcattagcaatgatgctgggctaactgaagtagttggaagtagtgctggaccaactgaatgtattgacttgaacaagacaccagcacggaaacccaagaagaaaaagcacaggccaaaggtgctaaaggacgataaaccatcgaagacacctaaatctgctactccaataccttcaacagaaaaggtagaaaaaccatctggaaagagaaaatatgtccgcaagaagacatctccaggccaacctcctgcagaacaggcagctagctcacactgcagatctgagctgaagtcagttaaacgaagtttggactttggtggagaagtactgcaagagagtacacaatctggatctcaagttccggtggcagaaatatgtactggtcccaagcgtcaatcaataccttctaccatccaaagagattcgcaaagccagttggcttgccacgtggtttctagcaccagctcaattcacacttcagctagtcagatggttaatgcacatttgtttcctcctgataacatgccaaatggagtattgcttgacctcaataattctactagtcagttacaaaacgaacatgctaaatttgtggacagtccggcacgtctttttggttccagaataagacagacatcaggtaaaaattctttgctagaaatctatgctggcatgtcagatagaaatgtacctgatctcaacagttcaatcagtcagacgcatagcatgtctactgattttgctcaatacttgctttcatcctcacaagcttctgtaagggaaacacaaatggccaatcagatgcttaatggtcataggatgccagaaaatccaattacacctagtcattgtattgaaagggctgcattgaaggaacatttgaatcatgttcctcacgcaaaagccgcagtgatgaatggccaaatgccccatagttacaggttggcgcaaaatcccatcctacctccaaatcatattgaagggtatcaagtgatggaaaatttgagtgaacttgtcacgacaaatgactatctaactgctagtcctttcagtcaaactggagctgcaaataggcagcataatattggtgactccatgcatatacatgcattggatcctagaagagagagtaatgcttcaagtggttcttggatatcattaggtgtgaactttaaccaacaaaataatggatgggcatctgcaggtgctgccgatgctgcgagctcacatgccccatatttttcagaacctcacaaaagaatgaggacagcttatcttaacaattatccaaatggagtcgtgggacatttttctacctcatctacggatttgtcaaataatgagaatgaaaatgtggcctcagcaatcaactcaaacgtttttacccttgctgatgcacaaagattgatagcccgtgagaaatcacgagcttcccaaagaatgatcagttttagatcatctaaaaatgatatggttaacagatcagaaatggtccatcaacatggcagacctgctccgcatggctctgcatgcagggagtctattgaagtacctgacaaacagttcgggctcatgacagaagaactcacacaattacctagtatgccaaataacccacaaagggaaaaatatattccgcaaactggaagttgccaacttcagtctttggaacatgacatggttaaagggcataacttggcaggtgaattgcataagcaagtaacttcacctcaagttgttattcagagcaatttctgtgttacccctcctgatgtgctcggcagaagaaccagtggggagcatttaagaacccttatagctccaacacatgcatcgacatgtaaggacactctgaaagctttaagttgtcaactggagagttctagagacattattaggcctcctgtcaatcctatagggccatcctctgccgatgttccaagaactgataaccatcaagtcaaggtttctgaagaaaccgttacagccaaactccctgagaagcgaaaagtaggacgtcccagaaaagagttaaaacctggtgagaaaccaaaacctagaggccgtccaaggaagggaaaagttgttggtggagaacttgcatcaaaggatagtcacactaatccattgcaaaatgagagtacttcatgttcttatggtccttatgcaggggaggcttctgttggaagagcagttaaagcaaatagagttggagaaaacatttctggagctatggtatccctactggattctttagatattgttattcaaaagataaaggtcttggacataaacaaatcagaagaccctgtgacagctgaacctcatggtgctcttgtcccttacaatggagaatttggtcctattgttccttttgaggggaaagtgaaaagaaaacgctctcgagccaaagtggatcttgaccctgtaactgctttaatgtggaagttactaatgggaccagatatgagtgattgtgctgaaggtatggataaggataaagagaaatggctaaatgaagaaagaaaaatattccaagggcgtgttgattcatttattgctcgaatgcatctagttcaaggagatcggcgtttttctccttggaaaggatcagttgtagattctgtagtgggagtatttcttacacagaatgtttcggaccatctttccagctctgcatttatggctcttgctgcaaaatttcctgtaaagccagaagcctctgaaaaacccgcaaatgtgatgtttcatacaatttcagaaaatggtgattgttctgggttgtttggtaattctgtcaagctacagggtgagatccttgttcaggaggccagcaacacagcagcctcttttatcacaaccgaggataaggaaggaagtaacagtgtggaattgcttggaagttcttttggggatggagtggatggtgcagcaggagtttattctaatatttatgagaatctgccagctagactgcatgctactaggcgtccagtcgttcaaactggaaacgctgtcgaagcggaagatgggtcactggagggtgttgtttcatcagaaaactccactatttcatctcaaaattcatcagattatctatttcacatgtctgatcatatgttttcgagcatgttactaaatttcactgccgaagacattggcagcagaaatatgcccaaagcaacaagaaccacatatacagaacttctacgaatgcaggagctgaagaacaagtctaatgaaaccattgaatcatcagagtatcatggggttccagtctcatgtagtaacaacattcaagtgctcaatggaatacaaaatatcggcagtaaacatcagcctttacattcctctatttcatatcaccagactggccaagttcacctcccagacatagtacatgcgagtgatttggagcaatcagtatacactggccttaatagagtgcttgattctaatgttacacaaaccagttattatccttcacctcatcctggaattgcctgtaacaatgaaacacaaaaggctgactctttaagcaacatgttatatggtatagatagatcagataagactacttccctgtctgagcctacaccaagaatcgataactgttttcaaccattaagttcagagaaaatgtcatttgctagggaacagtcctcttctgaaaattatctttcaaggaatgaagctgaagctgcatttgttaaacagcatggaacatcaaatgtgcaaggtgataatactgtcaggacagagcaaaatggaggtgaaaattctcaatcaggatacagccaacaggatgataatgttggatttcaaacagcgacaaccagtaatctttattcttcaaacttatgccaaaaccagaaagcaaattctgaagtactacacggagtttcttccaacttgatagagaattctaaagatgacaaaaagacttcccccaaagttccagtcgatggatcaaaagcaaagaggccaagagttggggctggtaaaaagaaaacatatgattgggatatgttgagaaaagaagttctttacagtcatggtaataaagaaagatcccagaatgctaaggactcaattgattgggaaacaataagacaagcagaggtgaaggaaatatctgacacaattagagagcgaggaatgaataacatgctggcagaacggataaaagacttcctaaaccgattggtgagagaccatgggagcatcgatcttgagtggttgcgctatgtcgattcagataaagcgaaggactatctcttaagcattagaggacttggacttaaaagtgttgagtgtgtgcgtcttttgacactccatcacatggcttttcctgtggatacaaatgttggtagaatatgtgtgaggcttggatgggtgccacttcagcccctacccgagtctcttcagttgcacctgttggagatgtatccaatgctggagaacatacagaaatacctctggccgaggttatgcaagcttgatcaacggacattgtatgagcttcactatcaaatgataacttttggaaaggtattttgtacaaaaagtaagcccaattgcaacgcatgcccaatgagagctgagtgcaagcactttgcaagtgcatttgccagtgcaaggctcgctcttcctggacctgaagagaagagtttagttacatctggaaccccaatagctgcagaaaccttccaccagacatatataagttctaggcctgtagtaagtcagcttgagtggaattcaaacacctgtcaccatggtatgaacaatcgccagccaatcattgaggagccagcaagcccagaacctgaacatgagacagaagagatgaaagagtgtgcaatagaggatagttttgtcgatgatccagaagaaatccctactatcaagcttaattttgaggagtttacacagaacctgaagagttatatgcaagcaaataacattgagattgaagatgctgatatgtcaaaggctttggtcgctataactcctgaagttgcttctatcccaactcctaagctcaagaatgtcagtcgcctaaggacagagcaccaagtctatgaactgccagattcacatccacttcttgaaggattcaaccaaagagaaccagatgatccttgcccatacctactctctatatggaccccaggtgaaacagctcaatcaactgatgcacctaagtcggtctgcaattcacaagagaatggtgaactatgtgcaagcaatacatgctttagttgcaacagtataagagaagcgcaggcccaaaaagttcgagggacactgctgataccatgccgaacagcaatgagaggaagctttccacttaatgggacatattttcaagtcaatgaggtatttgctgatcatgactcaagccggaacccgattgatgttccaaggagttggatatggaatctccctaggagaactgtttactttggaacttcaattccgacaatatttaaaggtttgacaactgaagaaatacaacattgcttttggagaggatttgtgtgcgtgagaggctttgataggacatcaagagcacccagaccactgtatgcaagactccactttccagcaagcaaaattaccaggaataaaaaatctgcaggttctgctccaggaagagatgatgaataggccatctggaaaaccagaaaggaaataaagaggaggtacatatgatctgccagaagatcactgacctgaaatggatcgctgaccaataagttgccgtaggcaattcaattatttctggccatatacatctgctgaaagttatgaactccagccactgacgaattcgtggtgctggtattcttcggcaacatgatccatcatacagattctatgcttggttgttgcaagcaattcttatgcggtgacagttgctgctgatagggagaaaaggcatgtccggcggctcagcggctctaactgtactttcatatgagtggaaccgattgttgtacatgtgaaaagtttgccattcaaaatggtcattcatgttgttaggtcattcatgtagtcgatgtcaaattaatcatcaattatttgatttgattcattcacaagtttaattggctctagatacttgtgagctgcaggccagcaatgtcataatgtatgtcgggaaaaggtagatataaatcgtcagcatttacctgaaatacccttcctctgtccataaatacaagggattttgggttgttaagcgtattttaagttcgatatgaaaattactttgatgttccg

SEQ ID NO: 9 - DNA, 16885 bp, Oryza sativa
agggcattgtagacattagcatttcaaacccagtaatccatgcctccaataataataagctaaaataaacaaggcctaagttaatcatgctaactcgtgctggctcaggcatgcgagtcctctagtcggactaggcacagttcgagcaacatggttggtcatggggcatcctatgcttgggccgctaccacggcacgtcacaacccggttgttatagcgggcctgacacaaagcatgcaagcatgcatgtcccagtccaacttcctttttttttcatatttttcatgtgggaatcaattttcttatggtttccctatatttttatgatttttctattttttttatggaccagtcaggccgatagatcgtccttggtgcatgggcctacttatgcctgggctatcacgacatgccctgtagcctccttgtgtcgtgcctaggttgaggcctcggcatgtgggcccgcacatgtcatgcaactgtggtgctcatgccatgctgggctgggccacccgtttcgacacaaatgaacgaagcgtaacgttaatgcatgcacttcttacactcactggagaggctcctagtttgcttagctgcctagcagcaaaagtcgcgttgtcctccatgtccggatcgaagcccatcatcaatgtatttagatcagagccacacgttgagctgcgcttcacgacgggaccaccgccaaaacacttgtttttcttccgtttaatattctagtttacaactttctataataaaatattaattcaaggttttaacattttagttgaaagttttaaaaattgtgttgaaacttttaaattttatactggaagtttcaaattttgtgttgtaagtttcaaactttggattgacttttttttagcaaatgttttaaatttgagttaaaagtttcaaatatgggtagtgtttttagattttgtactgaatgttttagaacttgagttgaaacttttagaatttaagttgagaattttaaattttgagttgaatgttttgaaattttgggttgagttttttaaactgtcgataaaaaaataaatttgagctaaaagtttcaaattttgagtagagtttttcaaatttgagttgattgttttaaaccattgaaaaagctggagcatgggaactcaagagttacgattcttttttttttcagggaaggggtgaattctattgattaaacagagtgattacaatcccgtaggacaatatcatgaatactaggaggagcatcaagtctccacactgcattattgctagtccttttggttaattgagctagttcatgagacactctattacaccctcttccaacatgatttagatggacttcaggaagtaaaccaacaaaactcctcgcttccaccaacaaggcacaccatcttgatttaggtcctctttgtttaggcttaggtttattggcctagacttttaagtcagcttattagcttatatgatttataagccggtggatttaatgtcctaagtttagtggttgagtcatacatctacctcacataagccaaaaaagcttctccaacctagcttttggcttaatagtgttagagtggcttatggcttcaaaaaagccaaacggaaaagctgcttgtttgtttaggcttagacttttcgacttataagttggcttataagcctaaacaaagaaagccttattttgcccaagggccatgagcttaatcacttctgagcaatcagtttcgaggataatagacatattgatccatttagccgataatgccaatccttctttgcacgccatgacttcaacttcttcgggctgaggtgctgtgaaaatgggtccgccgtgaggaaagaagtacttcccctctacaattcttgataaccactcccactccgacgtctcttgtttaaatctattcaaaatcacttcaaatatcgaattgctaaaaatgaacttattgtgctcatatttcaggtaggcccatccaaacccatcaagcgagctatagttatcgatgccacgcgtcaagcactcagctggcgtatgtgtgagggagatatttgaaagttggcaaaattacataaaccatcccatacccccattttgttatagaagcccacccaccgaacactaccagaccgagattgctctcttcatggatagttggttatgcccatattcttcaaatatgacaccaaatttagtgttaggggcaaaattgcataaacaaagttgatatggtactatgcgaatctacgttgaaaaaaatggaccgaatcagctactcactttgtgttgggtgggtagggtttttattttaacaaaatggattatcaagtggaatttcaaaacaaaatgactatgcaactccattccaatttatcatattgttcatgtgcgcaacatcgatggtgggagtggagtcactcagtctggactctgtagtggagttacttggtcacgtactcacatgacatatcttcaaatggatagctgattcggcctgtttctttaaatgtgataacaaataaagtgtcaaggcaaaatagcctatgccaattcactgtgaatccacgtcgaaagaaataagccaaattagccactcacatgtattggttgggtgggcttttaacaaaacaaacctcaaaacaaaatgattgagtgactccactccattttatcatattattcacgtgcaaggcagcggtggtgagagtgggggccactcaatctggactctagagtagagttactcagtcacatgagttattgttaaatgggtagttaatttggcctatttcttcaaatgcgacaacaaataaagtgtcaaggcaaaaaaaaacataaagcatatcttgctgcaaatccacgtcaaaagaaaataagccaaattagctacgtatgcgcattgtttgtgtgggggttttcaacaaaatgggttatcgtgtggatctcaaaacaaaatgactcagagtaactccgctctattttatcacattattcacgtgtaaggcagcgatggagagagtgaactatagtaaagttactcagtcgcacactcttaaatgaatagttgattccacccatttcttaaaatgtaacaacaaacaaagtgcccaggcaaaaatacacaaacccaaattagctacttatgtttattagttaggtgagttttacaacaaaataatatatcatacgaaatcccaaaacaaaatggctgagcgactccgttctattttatcacattattcacgtgtcggacagcgacggcggggcagtgaagtcactcagtctggactctctgaagtggagttactactcacgtgacgttactttttttgggaagtgtgtgcgctgcgatcagaagtagccaagcgtgcgcgaaatagcattcccgacgctcacctcccctccccccctccccccgcatcgttttctctcactctcctttcctcacttttcctctctctgaccgaatctctcccactcctctctactcctctcaaccctagctcgcctctaccctctctgctcatcgggcggcgcaggggaaggaaggcggcgtccggctgcgcggagcccggcgagggaggaggcggcgtcaggggggaccggcgcgggagggcggcgttcggcgttcggcgcggggggcggcggcgtccggccgactgcggcggcggctagatccggcgaaagaggctgcatcagcgccgattccccgactccccaaccctcaaacggtagcgaggtatactcggttgttttcccctcaggtctcaggctgatcagacgccgcactgccgatttccccctcgggcgagccatcggagcgggggccgttggctcccaaagcagacgcgagaattcactgaaattaccgcgccatcttatctccgcaagttgaagaatataattcgggcgcagtaatttttagtgaattcatgtgtctactactacatatgtctgcttgggagccaaccgcgtttcgatggctcgcctgaggggaaatcggcgggaggcgtttggtcagctttgctggtagtggggggaatttcacctaatgattgaatgatgggatatgctgggtaaaggaaggtatggttattttatattatctagaagagggtaaaaaagggagatggtcctttgggggctgtttgtcttgtttacatgggtttaggaaatattgcttaaatggatataaagttgaaaaatgtacttgagggaagttgtaggtgcacgtggggtcccacaatttttcttcactagtgcacctttagttatatattttttgcgcaagaggacaaaggcgctccgtgtaattttgagtaagggccggcgggatatttatttgtgtaaaggacctagccaagaaaagcatgatagtgcatatgtatcctttctttttcttttcttttgttttcataactgtcttacagaatttcatgttggctggtgacacttgtctcactcattatttggtatattttgactaaatgcaacgtgttggtgctcggtagtttatatttgtttttacgcattcttcattgactgtatgtatttgatgttgataccctgggctgtcttattttataggtggatgctgggaggccacataggaggcctgtgtgatccaagtgtgctgctcctgagttgaaattgcatagccatatagcaactactggtgtaaacttgagagatgaagtagtgaaaggaaatatgcaggattttggacaatggctgcctcaatctcagaccactgccgatctatatttctccagtattccaataccatcacagttcgatacttccatagagacgcagactagaacttctgcagttgtatcgtcagagaaagaatctgctaattcgttcgtccctcataatggtactgggcttgttgaacgcattagcaatgatgctgggctaactgaagtagttggaagtagtgctggaccaactgaatgtattgacttgaacaagacaccagcacggaaacccaagaagaaaaagcacaggccaaaggtgctaaaggacgataaaccatcgaagacacctaaatctgctactccaataccttcaacagaaaaggtagaaaaaccatctggaaagagaaaatatgtccgcaagaagacatctccaggccaacctcctgcagaacaggcagctagctcacactgcagatctgagctgaagtcagttaaacgaagtttggactttggtggagaagtactgcaagagagtacacaatctggatctcaagttccggtggcagaaatatgtactggtcccaagcgtcaatcaataccttctaccatccaaagagattcgcaaagccagttggcttgccacgtggtttctagcaccagctcaattcacacttcagctagtcagatggttaatgcacatttgtttcctcctgataacatgccaaatggagtattgcttgacctcaataattctactagtcagttacaaaacgaacatgctaaatttgtggacagtccggcacgtctttttggttccagaataagacagacatcaggtaaaaattctttgctagaaatctatgctggcatgtcagatagaaatgtacctgatctcaacagttcaatcagtcagacgcatagcatgtctactgattttgctcaatacttgctttcatcctcacaagcttctgtaagggaaacacaaatggccaatcagatgcttaatggtcataggatgccagaaaatccaattacacctagtcattgtattgaaagggctgcattgaaggaacatttgaatcatgttcctcacgcaaaagccgcagtgatgaatggccaaatgccccatagttacaggttggcgcaaaatcccatcctacctccaaatcatattgaagggtatcaagtgatggaaaatttgagtgaacttgtcacgacaaatgactatctaactgctagtcctttcagtcaaactggagctgcaaataggcagcataatattggtgactccatgcatatacatgcattggatcctagaagagagagtaatgcttcaagtggttcttggatatcattaggtgtgaactttaaccaacaaaataatggatgggcatctgcaggtgctgccgatgctgcgagctcacatgccccatatttttcagaacctcacaaaagaatgaggacagcttatcttaacaattatccaaatggagtcgtgggacatttttctacctcatctacggatttgtcaaataatgagaatgaaaatgtggcctcagcaatcaactcaaacgtttttacccttgctgatgcacaaagattgatagcccgtgagaaatcacgagcttcccaaagaatgatcagttttagatcatctaaaaatgatatggttaacagatcagaaatggtccatcaacatggcagacctgctccgcatggctctgcatgcagggagtctattgaagtacctgacaaacagttcgggctcatgacagaagaactcacacaattacctagtatgccaaataacccacaaagggaaaaatatattccgcaaactggaagttgccaacttcagtctttggaacatgacatggttaaagggcataacttggcaggtgaattgcataagcaagtaacttcacctcaagttgttattcagagcaatttctgtgttacccctcctgatgtgctcggcagaagaaccagtggggagcatttaagaacccttatagctccaacacatgcatcgacatgtaaggacactctgaaagctttaagttgtcaactggagagttctagagacattattaggcctcctgtcaatcctatagggccatcctctgccgatgttccaagaactgataaccatcaagtcaaggtttctgaagaaaccgttacagccaaactccctgagaagcgaaaagtaggacgtcccagaaaagagttaaaacctggtgagaaaccaaaacctagaggccgtccaaggaagggaaaagttgttggtggagaacttgcatcaaaggatagtcacactaatccattgcaaaatgagagtacttcatgttcttatggtccttatgcaggggaggcttctgttggaagagcagttaaagcaaatagagttggagaaaacatttctggagctatggtatccctactggattctttagatattgttattcaaaagataaaggtcttggacataaacaaatcagaagaccctgtgacagctgaacctcatggtgctcttgtcccttacaatggagaatttggtcctattgttccttttgaggggaaagtgaaaagaaaacgctctcgagccaaagtggatcttgaccctgtaactgctttaatgtggaagttactaatgggaccagatatgagtgattgtgctgaaggtatggataaggataaagagaaatggctaaatgaagaaagaaaaatattccaagggcgtgttgattcatttattgctcgaatgcatctagttcaaggtatttctatcattttaaaattgttttcctaacatgaacatgatggcttccatcttgtgattgctgccctcacattagtgaatggtctcaaatcttcaatatttactgtgtacccaaatcctatttcttcatcccaatatattcatgtttgtactcgtactgtcccattagacttgcattgtgctgtgaagatcaacacctttacttttaggattacctctatgtttgcaggagatcggcgtttttctccttggaaaggatcagttgtagattctgtagtgggagtatttcttacacagaatgtttcggaccatctttccaggtgaataatgcctagagcctatttgaaaactgtgacttgacttgcattgtgaggttatgttgtttttctgtctgactatttccttttttttcagctctgcatttatggctcttgctgcaaaatttcctgtaaagccagaagcctctgaaaaacccgcaaatgtgatgtttcatacaatttcagaaaatggtgattgttctgggttgtttggtaattctgtcaagctacagggtgagatccttgttcaggaggccagcaacacagcagcctcttttatcacaaccgaggataaggaaggaagtaacagtgtggaattgcttggaagttcttttggggatggagtggatggtgcagcaggagtttattctaatatttatgagaatctgccagctagactgcatgctactaggcgtccagtcgttcaaactggaaacgctgtcgaagcggaagatgggtcactggagggtgttgtttcatcagaaaactccactatttcatctcaaaattcatcagattatctatttcacatgtctgatcatatgttttcgagcatgttactaaatttcactgccgaagacattggcagcagaaatatgcccaaagcaacaagaaccacatatacagaacttctacgaatgcaggagctgaagaacaagtctaatgaaaccattgaatcatcagagtatcatggggttccagtctcatgtagtaacaacattcaagtgctcaatggaatacaaaatatcggcagtaaacatcagcctttacattcctctatttcatatcaccagactggccaagttcacctcccagacatagtacatgcgagtgatttggagcaatcagtatacactggccttaatagagtgcttgattctaatgttacacaaaccagttattatccttcacctcatcctggaattgcctgtaacaatgaaacacaaaaggctgactctttaagcaacatgttatatggtatagatagatcagataagactacttccctgtctgagcctacaccaagaatcgataactgttttcaaccattaagttcagagaaaatgtcatttgctagggaacagtcctcttctgaaaattatctttcaaggaatgaagctgaagctgcatttgttaaacagcatggaacatcaaatgtgcaaggtgataatactgtcaggacagagcaaaatggaggtgaaaattctcaatcaggatacagccaacaggatgataatgttggatttcaaacagcgacaaccagtaatctttattcttcaaacttatgccaaaaccagaaagcaaattctgaagtactacacggagtttcttccaacttgatagagaattctaaagatgacaaaaagacttcccccaaagttccagtcgatggatcaaaagcaaagaggccaagagttggggctggtaaaaagaaaacatatgattgggatatgttgagaaaagaagttctttacagtcatggtaataaagaaagatcccagaatgctaaggactcaattgattgggaaacaataagacaagcagaggtgaaggaaatatctgacacaattagagagcgaggaatgaataacatgctggcagaacggataaaagtaagtatggcataaaacagtttacattgaaagttgacataactctagtcatatgtgcatgcatgctattccatatagatttgcttatttgttggaattccaagttttggatcaaccatactcatctttagcaattcatgttgcaggacttcctaaaccgattggtgagagaccatgggagcatcgatcttgagtggttgcgctatgtcgattcagataaagcgaagtaagctaactaaatttattttgagcaaacattcataatgcaattggcccttgggcattctataatttgtcattttgacctctgcattgcttagcaatgacaattggatgtagtgagcatgggtaataatgtaagcaatgacaattggatgtagtgggcatggttaataattgaacatgtctgtgtttgcgggataataatgcctatcacctgtgagcctgtgacatgcaaaccttgaacgttgaaccttgaaccccctacctcgcactgtgtgctctcaaccaactgagcaagtgagggaccttgttgtatggaaaaaataattttaaataacccttgattcaaccaaagcttcataaaagaatatattttctattattcatttgaaccagcggttgaaccagtgaaccgatggtcttgctggtccggatttaataataactatggctagaacagattagagcaccgaatacttgcgcgatgctaaatatttcaatggggacacacctgctcgtgtgttgcatcaactacctaagccacacaggcatggcaatcaaatcagcttgcccatgtaacatcaactatctgatcgcgagaaggccggagctctcacttgatgtttgtcattcaaaaaatagttattcaccaatgcaatgtcaagctcccgtaaagaccatgaatgtagtttatccttctttgatcaagtttttatttatattaaagtgtttaccaatgtaatcctacattatttgtacctggtttttacatataaatacattgtaccttttgtgtttcttccagggactatctcttaagcattagaggacttggacttaaaagtgttgagtgtgtgcgtcttttgacactccatcacatggcttttcctgtatgtttcctttcacaaataattttcaagaatcttcgtttctttatttctggagaagtggagattttatctgtatctgttgatgatgtaggtggatacaaatgttggtagaatatgtgtgaggcttggatgggtgccacttcagcccctacccgagtctcttcagttgcacctgttggagatgtaagtatcttaaatccactggttggcttcactaatgctggagagtgataggagtttgatcatctgctattgaaggtatccaatgctggagaacatacagaaatacctctggccgaggttatgcaagcttgatcaacggacattgtgagttttagaaatgcagttaaaaactatatatataagagcatgtcattatctgagagtgtataacaggttcttgatgatatgtaggtatgagcttcactatcaaatgataacttttggaaaggtatgagacaacaactttgataaagtgaattcaacccaattactgtgttttgatggaccatctgtgttactttccttctaggtattttgtacaaaaagtaagcccaattgcaacgcatgcccaatgagagctgagtgcaagcactttgcaagtgcatttgccaggtaattctcaagatgtacatattttatatacattctgtgaaatcacggtgatgattgttaggtatgaacaattggctgagatcccccccctcccccctcccatccttttcctggtcctacaagttctcctaggctaatttaactggtgcataccacatttatgttattttgatacatcaaagattatgtttgtggttgtgaggctatattagtgtgttgtatgtaactcagttttgcaattgtagttttagttagaacacgttgttctctacattttaataaatactttttgactggacatcaatgactggtgtatttccgatataaaaaggttgattgttgccgagggatttcaattcggtccgaataggttcgacaaatgcagtgggcctattagtttaagagtgaaagttctatcagctgtttgactccactgtgacctttacactttgtacttttgaagaaacagactaacctgctcatattaaagtcttggaatgactccattgcgacctttacgctttgtattttagaagaaacagactaacctgttcatattagagtcttggaactgtgtgtgtgtgtgttttttttttttttgggggggggggggcatggagatttaatccaacattcctggatgaccttatattggtaatgatatggtttttttatgatatagtgcaaggctcgctcttcctggacctgaagagaagagtttagttacatctggaaccccaatagctgcagaaaccttccaccagacatatataagttctaggcctgtagtaagtcagcttgagtggaattcaaacacctgtcaccatggtatgaacaatcgccagccaatcattgaggagccagcaagcccagaacctgaacatgagacagaagagatgaaagagtgtgcaatagaggatagttttgtcgatgatccagaagaaatccctactatcaagcttaattttgaggagtttacacagaacctgaagagttatatgcaagcaaataacattgagattgaagatgctgatatgtcaaaggctttggtcgctataactcctgaagttgcttctatcccaactcctaagctcaagaatgtcagtcgcctaaggacagagcaccaagtgtatgatcttgtccctcttgcaaaaccaatctcatgaatatttactattgactatcatgtgttttgctgcattgcttacttctctgttttcaacatatatgtagctatgaactgccagattcacatccacttcttgaaggagtaagttcataaaacattatagaattctgtactttccttatcaccaactgagaatatattgatgcttattttcttacaatacacagttcaaccaaagagaaccagatgatccttgcccatacctactctctatatggaccccaggtaagaagtgcataaacagaacacaatatcatgggaaccaaacttttttcaatggttacttataattgttgaaatatgcaacaggtgaaacagctcaatcaactgatgcacctaagtcggtctgcaattcacaagagaatggtgaactatgtgcaagcaatacatgctttagttgcaacagtataagagaagcgcaggcccaaaaagttcgagggacactgctggtaagtagttgtttctgtaacatatgctcagttgcccttggttcaagatgtgctattcaagtttatcatgttcacgaatagtgataaagctgctatctgtcctagctattgtccaagctataacagttctgattcactggttgggcaccagctagggaataggatgtaaaaaacttatcccgcagtttgttgacaatctgtttttctttgttgaaaattaaaaatagataccatgccgaacagcaatgagaggaagctttccacttaatgggacatattttcaagtcaatgaggtgaaaacagaaagttcttaaagttgatcttagtttaattattataataccattaaaatatatgcaagtttctactttctagtatctcttttattagtgttcaaatgttatgcggcaggtatttgctgatcatgactcaagccggaacccgattgatgttccaaggagttggatatggaatctccctaggagaactgtttactttggaacttcaattccgacaatatttaaaggtatttcactaataaattttgaccaagaataggatttttggcagcgccaaatgtgccactatctttattgtgtgaagtccattatgtgattgtaataatttgaatcaccaagaggactaaggcctgctttgggacatattacgagcagcttttgcttgcaaagaaaccagattctggtgccgcaccttctccgctcttctgccacccaagtccgtccaatacccctcattgagcgcttggatcctaaccccatctgccatcatgcatcatcctgctaacaactgcttccaccattgcctgtttctgttgttgggaggcactcacgctgcttgctatagtttaggttttctttgtgtcctgatttagatggaatttccagctgctgtcttttacataactagctaaatgtccgcgctttgctatggataatagaaaatatattataatattgtcaaataaattaaatatgttttatacgaaatgtgttaacaatccttttgctatagggaatattgaccttaatttgattttatatgtggctatccatttagatttgtttgtttttctaataataataagttcaagggctaatgtacaaaattgacaatgggagtaggtggggtggcagattcactgccaccaccactaccttcttttaaaggggtatatagatttgcagcagtggttgcttgatctgtgatttgaaatgtcaagtacacgctcatgcatcagcaccatatgtctacgctcctgacccaacatgcaaccaatgcaattgagggttggctctgatacaattactaatgtcctatatccaaaacaactataggcctatgaccaaacataattaataacctcgcttgcgcttttgtcctcacttgctccatgtaaaagggttaacccgaggttactatgttaggaatagctgggtttatgaaacggttcaactctcaactcctcatatagcactaattcatgtattgctgtcagcagtgatttgagttccagatcatgctcataagataggaccaaattgtccttactatctactccctccgtcccaaaatataaggtatttccggtcaaaatatcttatattttgggatggagggagtactatactacggacccaccaccaaatagtgccgcagaagagagagagagagagagaagagggggtgggggtgggggtgtatgggtgaaataagaatagtgccaagtatttgccaacaaatgaggcggtcaaatgtgtcacatcaattgggaagtatgtcagatcaactgaaaatttgattgggaaattattattcatgcaacaaagctgtacaactgatcccatgtttctatcgcaggtttgacaactgaagaaatacaacattgcttttggagaggtaatcatttttttttgtatgtacgttttggtttccataacaaagagagatgaagtgtataggtactatgtttactgacaaggataataatagtagcaagtatataggcagaggagcatgtctctattctaccagtattattactcataataactagtatatccttttttttgccatttcagctgatagctactctccagtcaaaatatttgccatctctattgaacttttcattgtcttctgaatgtatcttactcttggatcattaatatttcattttgtcacgatatagtggtataggacaataaaatcatgggaagtatttattttcatcaccaatctactcatataattttcaaatgacaattataaatatcttaaaaatatattgttagttgtcctgtataaaataattgtcacaccctagtccacagcgacaagaatttgtgtctacaggctagagtgagtactctagaagtatcttcataggaatcggaataaaatgccaatgtgaatgaacaaggatatcaagtataccctcaaaatctctagagaggattgcgtaaatatgtaggtgtaattaaacaattgtttcatatggagggttttcttaaaggaggtacaagacttatcaatatgggtaaagtagtttttatccataggcattgttggcagaaagctgcttagggtagaatgctactccctccgtcccacaatataagagattttgagtttttgcttgcaacgtttgaccactcggcttattcaaaaatttttgaaattattatttattttatttgtgacttactttattattcacagtactttaagtacaacttttcgttttttatatttgcaaaaaaaattgtataagacgagtggtcaaacgttgtacgcaaaaactcaaaatcccttatattgtgggacggagggagtacttatggatgccttttttgtccaagatgtcagtaacattttctttcagggatgtggatttttacttcttttttccctaactttttcaggatttgtgtgcgtgagaggctttgataggacatcaagagcacccagaccactgtatgcaagactccactttccagcaagcaaaattaccaggaataaaaaatctgcaggttctgctccaggaagagatgatgaataggccatctggaaaaccagaaaggaaataaagaggaggtacatatgatctgccagaagatcactgacctgaaatggatcgctgaccaataagttgccgtaggcaattcaattatttctggccatatacatctgctgaaagttatgaactccagccactgacgaattcgtggtgctggtattcttcggcaacatgatccatcatacagattctatgcttggttgttgcaagcaattcttatgcggtgacagttgctgctgatagggagaaaaggcatgtccggcggctcagcggctctaactgtactttcatatgagtggaaccgattgttgtacatgtgaaaagtttgccattcaaaatggtcattcatgttgttaggtcattcatgtagtcgatgtcaaattaatcatcaattatttgatttgattcattcacaagtttaattggctctagatacttgtgagctgcaggccagcaatgtcataatgtatgtcgggaaaaggtagatataaatcgtcagcatttacctgaaatacccttcctctgtccataaatacaagggattttgggttgttaagcgtattttaagttcgatatgaaaattactttgatgttccgaagggcttattttgtcttgggttgtttagcatgtcataaggttgatattaaattactttcatgcccttaggagttttggaaagttgacgcttaacagatgcgactagcagtaagcaataaatgtctagatggattgagaaagtagtatttcttccgtctcaaaatattgctataagctctgtttgttagggttctaacttctaaattactttagaagttaggtatatagtgaagttgtggaactatttaaatatagttatatctctctagtttattttttattttatgagagcacttcaattcattccactctttttttttttggaattgaaatcatttggttgtgcttcagttctagaaaatgtggagctagagttgaagacgtgttaaacgggtcctta

SEQ ID NO: 10 - DNA, 35 bp, Oryza sativa
caatgaggtatttgctgatcatgactcaagccgga

SEQ ID NO: 11 - DNA, 56 bp, Oryza sativa
caatgagtgttcaaatgttatgcggcaggtatttgctgatcatgactcaagccgga

SEQ ID NO: 12 - protein, 152 aa, Oryza sativa
CNSQENGELCASNTCFSCNSIREAQAQKVRGTLLIPCRTAMRGSFPLNGTYFQVNEVFADHDSSRNPIDVPRSWIWNLPRRTVYFGTSIPTIFKGLTTEEIQHCFWRGFVCVRGFDRTSRAPRPLYARLHFPASKITRNKKSAGSAPGRDDE

SEQ ID NO: 13 - protein, 159 aa, Oryza sativa
CNSQENGELCASNTCFSCNSIREAQAQKVRGTLLIPCRTAMRGSFPLNGTYFQVNECSNVMRQVFADHDSSRNPIDVPRSWIWNLPRRTVYFGTSIPTIFKGLTTEEIQHCFWRGFVCVRGFDRTSRAPRPLYARLHFPASKITRNKKSAGSAPGRDDE

SEQ ID NO: 14 - protein, 7 aa, Oryza sativa
CSNVMRQ

SEQ ID NO: 15 - DNA, 19 bp, Artificial Sequence
  oligonucleotide primer
tgagtagttgcgttgttct

SEQ ID NO: 16 - DNA, 18 bp, Artificial Sequence
  oligonucleotide primer
tcttagtgagccgtttct

SEQ ID NO: 17 - DNA, 18 bp, Artificial Sequence
  oligonucleotide primer
ccttctgtgctatgggtt

SEQ ID NO: 18 - DNA, 18 bp, Artificial Sequence
  oligonucleotide primer
catgccaagacaccactt

SEQ ID NO: 19 - DNA, 18 bp, Artificial Sequence
  oligonucleotide primer
tggctttggaaacggtag

SEQ ID NO: 20 - DNA, 19 bp, Artificial Sequence
  oligonucleotide primer
tttagagggatgtgcgtca

SEQ ID NO: 21 - DNA, 18 bp, Artificial Sequence
  oligonucleotide primer
aaacaacgatccagcaaa

SEQ ID NO: 22 - DNA, 19 bp, Artificial Sequence
  oligonucleotide primer
ttggcaccgtattactttc

SEQ ID NO: 23 - DNA, 24 bp, Artificial Sequence
  oligonucleotide primer
acgcattcttcattgactgtatgt

SEQ ID NO: 24 - DNA, 24 bp, Artificial Sequence
  oligonucleotide primer
gccctttcaatacaatgactaggt

SEQ ID NO: 25 - DNA, 24 bp, Artificial Sequence
  oligonucleotide primer
gaacatttgaatcatgttcctcac

SEQ ID NO: 26 - DNA, 24 bp, Artificial Sequence
  oligonucleotide primer
actatcctttgatgcaagttctcc

SEQ ID NO: 27 - DNA, 24 bp, Artificial Sequence
  oligonucleotide primer
gttggaagagcagttaaagcaaat

SEQ ID NO: 28 - DNA, 24 bp, Artificial Sequence
  oligonucleotide primer
cttcggcagtgaaatttagtaaca

SEQ ID NO: 29 - DNA, 24 bp, Artificial Sequence
  oligonucleotide primer
tacagaacttctacgaatgcagga

SEQ ID NO: 30 - DNA, 24 bp, Artificial Sequence
  oligonucleotide primer
gcaacatgaattgctaaagatgag

SEQ ID NO: 31 - DNA, 35 bp, Artificial Sequence
  oligonucleotide primer
ctatacctcctcaactccggtcaccgtctccggcg

SEQ ID NO: 32 - DNA, 35 bp, Artificial Sequence; identical to SEQ ID NO: 31
  oligonucleotide primer
  C (18)..(18): 5-methylcytosine

SEQ ID NO: 33 - DNA, 35 bp, Artificial Sequence; identical to SEQ ID NO: 31
  oligonucleotide primer
  C (17)..(17): 5-methylcytosine

SEQ ID NO: 34 - DNA, 35 bp, Artificial Sequence; identical to SEQ ID NO: 31
  oligonucleotide primer
  C (22)..(22): 5-methylcytosine

SEQ ID NO: 35 - DNA, 34 bp, Artificial Sequence
  oligonucleotide primer
  g (18)..(18): abasic site
ctatacctcctcaactcggtcaccgtctccggcg

SEQ ID NO: 36 - DNA, 34 bp, Artificial Sequence; identical to SEQ ID NO: 35
  oligonucleotide primer
  C (17)..(17): abasic site

SEQ ID NO: 37 - DNA, 34 bp, Artificial Sequence
  oligonucleotide primer
  T (15)..(15): abasic site
ctatacctcctcaatccggtcaccgtctccggcg

SEQ ID NO: 38 - DNA, 34 bp, Artificial Sequence
  oligonucleotide primer
  A (12)..(12): abasic site
ctatacctcctaactccggtcaccgtctccggcg

SEQ ID NO: 39 - DNA, 35 bp, Artificial Sequence
  oligonucleotide primer
ctatacctcctcaactctggtcaccgtctccggcg

SEQ ID NO: 40 - DNA, 35 bp, Artificial Sequence
  oligonucleotide primer
cgccggagacggtgaccggagttgaggaggtatag

SEQ ID NO: 41 - DNA, 35 bp, Artificial Sequence; identical to SEQ ID NO: 40
  oligonucleotide primer
  C (17)..(17): 5-methylcytosine

SEQ ID NO: 42 - DNA, 31 bp, Artificial Sequence
  oligonucleotide primer
ttaatctagaatgcagagcattatggactcg

SEQ ID NO: 43 - DNA, 34 bp, Artificial Sequence
  oligonucleotide primer
cggtcgacttaggttttgttgttcttcaatttgc

SEQ ID NO: 44 - protein, 22 aa, Artificial Sequence
  Motif
DHGSIDLEWLRDHGSIDLEWLR

SEQ ID NO: 45 - protein, 17 aa, Artificial Sequence
  Motif
GLGLKSVECVRLLTLHH

SEQ ID NO: 46 - protein, 11 aa, Artificial Sequence
  Motif
AFPVDTNVGRI

SEQ ID NO: 47 - protein, 21 aa, Artificial Sequence
  Motif
VRLGWVPLQPLPESLQLHLLE

SEQ ID NO: 48 - protein, 22 aa, Artificial Sequence
  Motif
ELHYQMITFGKVFCTKSKPNCN

SEQ ID NO: 49 - protein, 14 aa, Artificial Sequence
  Motif
HFASAFASARLALP

SEQ ID NO: 50 - protein, 1393 aa, Arabidopsis thaliana
MEKQRREESSFQQPPWIPQTPMKPFSPICPYTVEDQYHSSQLEERRFVGNKDMSGLDHLSFGDLLALANTASLIFSGQTPIPTRNTEVMQKGTEEVESLSSVSNNVAEQILKTPEKPKRKKHRPKVRREAKPKREPKPRAPRKSVVTDGQESKTPKRKYVRKKVEVSKDQDATPVESSAAVETSTRPKRLCRRVLDFEAENGENQTNGDIREAGEMESALQEKQLDSGNQELKDCLLSAPSTPKRKRSQGKRKGVQPKKNGSNLEEVDISMAQAAKRRQGPTCCDMNLSGIQYDEQCDYQKMHWLYSPNLQQGGMRYDAICSKVFSGQQHNYVSAFHATCYSSTSQLSANRVLTVEERREGIFQGRQESELNVLSDKIDTPIKKKTTGHARFRNLSSMNKLVEVPEHLTSGYCSKPQQNNKILVDTRVTVSKKKPTKSEKSQTKQKNLLPNLCRFPPSFTGLSPDELWKRRNSIETISELLRLLDINREHSETALVPYTMNSQIVLFGGGAGAIVPVTPVKKPRPRPKVDLDDETDRVWKLLLENINSEGVDGSDEQKAKWWEEERNVFRGRADSFIARMHLVQGDRRFTPWKGSVVDSVVGVFLTQNVSDHLSSSAFMSLASQFPVPFVPSSNFDAGTSSMPSIQITYLDSEETMSSPPDHNHSSVTLKNTQPDEEKDYVPSNETSRSSSEIAISAHESVDKTTDSKEYVDSDRKGSSVEVDKTDEKCRVLNLFPSEDSALTCQHSMVSDAPQNTERAGSSSEIDLEGEYRTSFMKLLQGVQVSLEDSNQVSPNMSPGDCSSEIKGFQSMKEPTKSSVDSSEPGCCSQQDGDVLSCQKPTLKEKGKKVLKEEKKAFDWDCLRREAQARAGIREKTRSTMDTVDWKAIRAADVKEVAETIKSRGMNHKLAERIQGFLDRLVNDHGSIDLEWLRDVPPDKAKEYLLSFNGLGLKSVECVRLLTLHHLAFPVDTNVGRIAVRLGWVPLQPLPESLQLHLLEMYPMLESIQKYLWPRLCKLDQKTLYELHYQMITFGKVFCTKSKPNCNACPMKGECRHFASAFASARLALPSTEKGMGTPDKNPLPLHLPEPFQREQGSEVVQHSEPAKKVTCCEPIIEEPASPEPETAEVSIADIEEAFFEDPEEIPTIRLNMDAFTSNLKKIMEHNKELQDGNMSSALVALTAETASLPMPKLKNISQLRTEHRVYELPDEHPLLAQLEKREPDDPCSYLLAIWTPGETADSIQPSVSTCIFQANGMLCDEETCFSCNSIKETRSQIVRGTILIPCRTAMRGSFPLNGTYFQVNEVFADHASSLNPINVPRELIWELPRRTVYFGTSVPTIFKGLSTEKIQACFWKGYVCVRGFDRKTRGPKPLIARLHFPASKLKGQQANLA